European Patent Specification EP 3 587 587 B1, published November 6, 2024. Title: COMPOSITIONS AND METHODS FOR QUANTIFYING A NUCLEIC ACID SEQUENCE IN A SAMPLE. Applicant: ENVIROLOGIX INC., et al. The sequence listing filed with the application follows.

SEQUENCE LISTING (61 sequences)

SEQ ID NO: 1 - DNA, 33 bp, Artificial Sequence
  source: /note="Description of Artificial Sequence: Synthetic oligonucleotide"
  source: /note="Description of Combined DNA/RNA Molecule: Synthetic oligonucleotide"
  modified_base (22)..(22): 2'-O-methyl modified RNA base
tgactccatatggagtcacatggttcattcgtg

SEQ ID NO: 2 - DNA, 33 bp, Artificial Sequence; identical to SEQ ID NO: 1
  source: /note="Description of Artificial Sequence: Synthetic oligonucleotide"
  source: /note="Description of Combined DNA/RNA Molecule: Synthetic oligonucleotide"
  modified_base (23)..(23): 2'-O-methyl modified RNA base

SEQ ID NO: 3 - DNA, 33 bp, Artificial Sequence
  source: /note="Description of Artificial Sequence: Synthetic oligonucleotide"
  source: /note="Description of Combined DNA/RNA Molecule: Synthetic oligonucleotide"
  modified_base (24)..(24): 2'-O-methyl modified RNA base
tgactccatatggagtcacatggutcattcgtg

SEQ ID NO: 4 - DNA, 33 bp, Artificial Sequence
  source: /note="Description of Artificial Sequence: Synthetic oligonucleotide"
  source: /note="Description of Combined DNA/RNA Molecule: Synthetic oligonucleotide"
  modified_base (25)..(25): 2'-O-methyl modified RNA base
tgactccatatggagtcacatggtucattcgtg

SEQ ID NO: 5 - DNA, 33 bp, Artificial Sequence; identical to SEQ ID NO: 1
  source: /note="Description of Artificial Sequence: Synthetic oligonucleotide"
  source: /note="Description of Combined DNA/RNA Molecule: Synthetic oligonucleotide"
  modified_base (26)..(26): 2'-O-methyl modified RNA base

SEQ ID NO: 6 - DNA, 33 bp, Artificial Sequence; identical to SEQ ID NO: 1
  source: /note="Description of Artificial Sequence: Synthetic oligonucleotide"
  source: /note="Description of Combined DNA/RNA Molecule: Synthetic oligonucleotide"
  modified_base (27)..(27): 2'-O-methyl modified RNA base

SEQ ID NO: 7 - DNA, 33 bp, Artificial Sequence
  source: /note="Description of Artificial Sequence: Synthetic oligonucleotide"
  source: /note="Description of Combined DNA/RNA Molecule: Synthetic oligonucleotide"
  modified_base (28)..(28): 2'-O-methyl modified RNA base
tgactccatatggagtcacatggttcautcgtg

SEQ ID NO: 8 - DNA, 33 bp, Artificial Sequence
  source: /note="Description of Artificial Sequence: Synthetic oligonucleotide"
  source: /note="Description of Combined DNA/RNA Molecule: Synthetic oligonucleotide"
  modified_base (29)..(29): 2'-O-methyl modified RNA base
tgactccatatggagtcacatggttcatucgtg

SEQ ID NO: 9 - DNA, 33 bp, Artificial Sequence; identical to SEQ ID NO: 1
  source: /note="Description of Artificial Sequence: Synthetic oligonucleotide"
  source: /note="Description of Combined DNA/RNA Molecule: Synthetic oligonucleotide"
  modified_base (30)..(30): 2'-O-methyl modified RNA base

SEQ ID NO: 10 - DNA, 33 bp, Artificial Sequence; identical to SEQ ID NO: 1
  source: /note="Description of Artificial Sequence: Synthetic oligonucleotide"
  source: /note="Description of Combined DNA/RNA Molecule: Synthetic oligonucleotide"
  modified_base (31)..(31): 2'-O-methyl modified RNA base

SEQ ID NO: 11 - DNA, 33 bp, Artificial Sequence
  source: /note="Description of Artificial Sequence: Synthetic oligonucleotide"
  source: /note="Description of Combined DNA/RNA Molecule: Synthetic oligonucleotide"
  modified_base (32)..(32): 2'-O-methyl modified RNA base
tgactccatatggagtcacatggttcattcgug

SEQ ID NO: 12 - DNA, 33 bp, Artificial Sequence; identical to SEQ ID NO: 1
  source: /note="Description of Artificial Sequence: Synthetic oligonucleotide"
  source: /note="Description of Combined DNA/RNA Molecule: Synthetic oligonucleotide"
  modified_base (33)..(33): 2'-O-methyl modified RNA base

SEQ ID NO: 13 - DNA, 33 bp, Artificial Sequence; identical to SEQ ID NO: 1
  source: /note="Description of Artificial Sequence: Synthetic oligonucleotide"
  source: /note="Description of Combined DNA/RNA Molecule: Synthetic oligonucleotide"
  modified_base (22)..(23): 2'-O-methyl modified RNA base

SEQ ID NO: 14 - DNA, 33 bp, Artificial Sequence; identical to SEQ ID NO: 3
  source: /note="Description of Artificial Sequence: Synthetic oligonucleotide"
  source: /note="Description of Combined DNA/RNA Molecule: Synthetic oligonucleotide"
  modified_base (23)..(24): 2'-O-methyl modified RNA base

SEQ ID NO: 15 - DNA, 33 bp, Artificial Sequence
  source: /note="Description of Artificial Sequence: Synthetic oligonucleotide"
  source: /note="Description of Combined DNA/RNA Molecule: Synthetic oligonucleotide"
  modified_base (24)..(25): 2'-O-methyl modified RNA base
tgactccatatggagtcacatgguucattcgtg

SEQ ID NO: 16 - DNA, 33 bp, Artificial Sequence; identical to SEQ ID NO: 4
  source: /note="Description of Artificial Sequence: Synthetic oligonucleotide"
  source: /note="Description of Combined DNA/RNA Molecule: Synthetic oligonucleotide"
  modified_base (25)..(26): 2'-O-methyl modified RNA base

SEQ ID NO: 17 - DNA, 33 bp, Artificial Sequence; identical to SEQ ID NO: 1
  source: /note="Description of Artificial Sequence: Synthetic oligonucleotide"
  source: /note="Description of Combined DNA/RNA Molecule: Synthetic oligonucleotide"
  modified_base (26)..(27): 2'-O-methyl modified RNA base

SEQ ID NO: 18 - DNA, 33 bp, Artificial Sequence; identical to SEQ ID NO: 7
  source: /note="Description of Artificial Sequence: Synthetic oligonucleotide"
  source: /note="Description of Combined DNA/RNA Molecule: Synthetic oligonucleotide"
  modified_base (27)..(28): 2'-O-methyl modified RNA base

SEQ ID NO: 19 - DNA, 33 bp, Artificial Sequence
  source: /note="Description of Artificial Sequence: Synthetic oligonucleotide"
  source: /note="Description of Combined DNA/RNA Molecule: Synthetic oligonucleotide"
  modified_base (28)..(29): 2'-O-methyl modified RNA base
tgactccatatggagtcacatggttcauucgtg

SEQ ID NO: 20 - DNA, 33 bp, Artificial Sequence; identical to SEQ ID NO: 8
  source: /note="Description of Artificial Sequence: Synthetic oligonucleotide"
  source: /note="Description of Combined DNA/RNA Molecule: Synthetic oligonucleotide"
  modified_base (29)..(30): 2'-O-methyl modified RNA base

SEQ ID NO: 21 - DNA, 33 bp, Artificial Sequence; identical to SEQ ID NO: 1
  source: /note="Description of Artificial Sequence: Synthetic oligonucleotide"
  source: /note="Description of Combined DNA/RNA Molecule: Synthetic oligonucleotide"
  modified_base (30)..(31): 2'-O-methyl modified RNA base

SEQ ID NO: 22 - DNA, 33 bp, Artificial Sequence; identical to SEQ ID NO: 11
  source: /note="Description of Artificial Sequence: Synthetic oligonucleotide"
  source: /note="Description of Combined DNA/RNA Molecule: Synthetic oligonucleotide"
  modified_base (31)..(32): 2'-O-methyl modified RNA base

SEQ ID NO: 23 - DNA, 33 bp, Artificial Sequence; identical to SEQ ID NO: 11
  source: /note="Description of Artificial Sequence: Synthetic oligonucleotide"
  source: /note="Description of Combined DNA/RNA Molecule: Synthetic oligonucleotide"
  modified_base (32)..(33): 2'-O-methyl modified RNA base

SEQ ID NO: 24 - DNA, 33 bp, Artificial Sequence; identical to SEQ ID NO: 3
  source: /note="Description of Artificial Sequence: Synthetic oligonucleotide"
  source: /note="Description of Combined DNA/RNA Molecule: Synthetic oligonucleotide"
  modified_base (22)..(24): 2'-O-methyl modified RNA base

SEQ ID NO: 25 - DNA, 33 bp, Artificial Sequence; identical to SEQ ID NO: 15
  source: /note="Description of Artificial Sequence: Synthetic oligonucleotide"
  source: /note="Description of Combined DNA/RNA Molecule: Synthetic oligonucleotide"
  modified_base (23)..(25): 2'-O-methyl modified RNA base

SEQ ID NO: 26 - DNA, 33 bp, Artificial Sequence; identical to SEQ ID NO: 15
  source: /note="Description of Artificial Sequence: Synthetic oligonucleotide"
  source: /note="Description of Combined DNA/RNA Molecule: Synthetic oligonucleotide"
  modified_base (24)..(26): 2'-O-methyl modified RNA base

SEQ ID NO: 27 - DNA, 33 bp, Artificial Sequence; identical to SEQ ID NO: 4
  source: /note="Description of Artificial Sequence: Synthetic oligonucleotide"
  source: /note="Description of Combined DNA/RNA Molecule: Synthetic oligonucleotide"
  modified_base (25)..(27): 2'-O-methyl modified RNA base

SEQ ID NO: 28 - DNA, 33 bp, Artificial Sequence; identical to SEQ ID NO: 7
  source: /note="Description of Artificial Sequence: Synthetic oligonucleotide"
  source: /note="Description of Combined DNA/RNA Molecule: Synthetic oligonucleotide"
  modified_base (26)..(28): 2'-O-methyl modified RNA base

SEQ ID NO: 29 - DNA, 33 bp, Artificial Sequence; identical to SEQ ID NO: 19
  source: /note="Description of Artificial Sequence: Synthetic oligonucleotide"
  source: /note="Description of Combined DNA/RNA Molecule: Synthetic oligonucleotide"
  modified_base (27)..(29): 2'-O-methyl modified RNA base

SEQ ID NO: 30 - DNA, 33 bp, Artificial Sequence; identical to SEQ ID NO: 19
  source: /note="Description of Artificial Sequence: Synthetic oligonucleotide"
  source: /note="Description of Combined DNA/RNA Molecule: Synthetic oligonucleotide"
  modified_base (28)..(30): 2'-O-methyl modified RNA base

SEQ ID NO: 31 - DNA, 33 bp, Artificial Sequence; identical to SEQ ID NO: 8
  source: /note="Description of Artificial Sequence: Synthetic oligonucleotide"
  source: /note="Description of Combined DNA/RNA Molecule: Synthetic oligonucleotide"
  modified_base (29)..(31): 2'-O-methyl modified RNA base

SEQ ID NO: 32 - DNA, 33 bp, Artificial Sequence; identical to SEQ ID NO: 11
  source: /note="Description of Artificial Sequence: Synthetic oligonucleotide"
  source: /note="Description of Combined DNA/RNA Molecule: Synthetic oligonucleotide"
  modified_base (30)..(32): 2'-O-methyl modified RNA base

SEQ ID NO: 33 - DNA, 33 bp, Artificial Sequence; identical to SEQ ID NO: 11
  source: /note="Description of Artificial Sequence: Synthetic oligonucleotide"
  source: /note="Description of Combined DNA/RNA Molecule: Synthetic oligonucleotide"
  modified_base (31)..(33): 2'-O-methyl modified RNA base

SEQ ID NO: 34 - DNA, 33 bp, Artificial Sequence; identical to SEQ ID NO: 15
  source: /note="Description of Artificial Sequence: Synthetic oligonucleotide"
  source: /note="Description of Combined DNA/RNA Molecule: Synthetic oligonucleotide"
  modified_base (22)..(25): 2'-O-methyl modified RNA base

SEQ ID NO: 35 - DNA, 33 bp, Artificial Sequence; identical to SEQ ID NO: 15
  source: /note="Description of Artificial Sequence: Synthetic oligonucleotide"
  source: /note="Description of Combined DNA/RNA Molecule: Synthetic oligonucleotide"
  modified_base (23)..(26): 2'-O-methyl modified RNA base

SEQ ID NO: 36 - DNA, 33 bp, Artificial Sequence; identical to SEQ ID NO: 15
  source: /note="Description of Artificial Sequence: Synthetic oligonucleotide"
  source: /note="Description of Combined DNA/RNA Molecule: Synthetic oligonucleotide"
  modified_base (24)..(27): 2'-O-methyl modified RNA base

SEQ ID NO: 37 - DNA, 33 bp, Artificial Sequence
  source: /note="Description of Artificial Sequence: Synthetic oligonucleotide"
  source: /note="Description of Combined DNA/RNA Molecule: Synthetic oligonucleotide"
  modified_base (25)..(28): 2'-O-methyl modified RNA base
tgactccatatggagtcacatggtucautcgtg

SEQ ID NO: 38 - DNA, 33 bp, Artificial Sequence; identical to SEQ ID NO: 19
  source: /note="Description of Artificial Sequence: Synthetic oligonucleotide"
  source: /note="Description of Combined DNA/RNA Molecule: Synthetic oligonucleotide"
  modified_base (26)..(29): 2'-O-methyl modified RNA base

SEQ ID NO: 39 - DNA, 33 bp, Artificial Sequence; identical to SEQ ID NO: 19
  source: /note="Description of Artificial Sequence: Synthetic oligonucleotide"
  source: /note="Description of Combined DNA/RNA Molecule: Synthetic oligonucleotide"
  modified_base (27)..(30): 2'-O-methyl modified RNA base

SEQ ID NO: 40 - DNA, 33 bp, Artificial Sequence; identical to SEQ ID NO: 19
  source: /note="Description of Artificial Sequence: Synthetic oligonucleotide"
  source: /note="Description of Combined DNA/RNA Molecule: Synthetic oligonucleotide"
  modified_base (28)..(31): 2'-O-methyl modified RNA base

SEQ ID NO: 41 - DNA, 33 bp, Artificial Sequence
  source: /note="Description of Artificial Sequence: Synthetic oligonucleotide"
  source: /note="Description of Combined DNA/RNA Molecule: Synthetic oligonucleotide"
  modified_base (29)..(32): 2'-O-methyl modified RNA base
tgactccatatggagtcacatggttcatucgug

SEQ ID NO: 42 - DNA, 33 bp, Artificial Sequence; identical to SEQ ID NO: 11
  source: /note="Description of Artificial Sequence: Synthetic oligonucleotide"
  source: /note="Description of Combined DNA/RNA Molecule: Synthetic oligonucleotide"
  modified_base (30)..(33): 2'-O-methyl modified RNA base

SEQ ID NO: 43 - DNA, 33 bp, Artificial Sequence; identical to SEQ ID NO: 15
  source: /note="Description of Artificial Sequence: Synthetic oligonucleotide"
  source: /note="Description of Combined DNA/RNA Molecule: Synthetic oligonucleotide"
  modified_base (22)..(26): 2'-O-methyl modified RNA base

SEQ ID NO: 44 - DNA, 33 bp, Artificial Sequence; identical to SEQ ID NO: 15
  source: /note="Description of Artificial Sequence: Synthetic oligonucleotide"
  source: /note="Description of Combined DNA/RNA Molecule: Synthetic oligonucleotide"
  modified_base (23)..(27): 2'-O-methyl modified RNA base

SEQ ID NO: 45 - DNA, 33 bp, Artificial Sequence
  source: /note="Description of Artificial Sequence: Synthetic oligonucleotide"
  source: /note="Description of Combined DNA/RNA Molecule: Synthetic oligonucleotide"
  modified_base (24)..(28): 2'-O-methyl modified RNA base
tgactccatatggagtcacatgguucautcgtg

SEQ ID NO: 46 - DNA, 33 bp, Artificial Sequence
  source: /note="Description of Artificial Sequence: Synthetic oligonucleotide"
  source: /note="Description of Combined DNA/RNA Molecule: Synthetic oligonucleotide"
  modified_base (25)..(29): 2'-O-methyl modified RNA base
tgactccatatggagtcacatggtucauucgtg

SEQ ID NO: 47 - DNA, 33 bp, Artificial Sequence; identical to SEQ ID NO: 19
  source: /note="Description of Artificial Sequence: Synthetic oligonucleotide"
  source: /note="Description of Combined DNA/RNA Molecule: Synthetic oligonucleotide"
  modified_base (26)..(30): 2'-O-methyl modified RNA base

SEQ ID NO: 48 - DNA, 33 bp, Artificial Sequence; identical to SEQ ID NO: 19
  source: /note="Description of Artificial Sequence: Synthetic oligonucleotide"
  source: /note="Description of Combined DNA/RNA Molecule: Synthetic oligonucleotide"
  modified_base (27)..(31): 2'-O-methyl modified RNA base

SEQ ID NO: 49 - DNA, 33 bp, Artificial Sequence
  source: /note="Description of Artificial Sequence: Synthetic oligonucleotide"
  source: /note="Description of Combined DNA/RNA Molecule: Synthetic oligonucleotide"
  modified_base (28)..(32): 2'-O-methyl modified RNA base
tgactccatatggagtcacatggttcauucgug

SEQ ID NO: 50 - DNA, 33 bp, Artificial Sequence; identical to SEQ ID NO: 41
  source: /note="Description of Artificial Sequence: Synthetic oligonucleotide"
  source: /note="Description of Combined DNA/RNA Molecule: Synthetic oligonucleotide"
  modified_base (29)..(33): 2'-O-methyl modified RNA base

SEQ ID NO: 51 - DNA, 33 bp, Artificial Sequence
  source: /note="Description of Artificial Sequence: Synthetic oligonucleotide"
  source: /note="Description of Combined DNA/RNA Molecule: Synthetic oligonucleotide"
  modified_base (22)..(33): 2'-O-methyl modified RNA base
tgactccatatggagtcacatgguucauucgug

SEQ ID NO: 52 - DNA, 33 bp, Artificial Sequence; identical to SEQ ID NO: 51
  source: /note="Description of Artificial Sequence: Synthetic oligonucleotide"
  source: /note="Description of Combined DNA/RNA Molecule: Synthetic oligonucleotide"
  modified_base (23)..(33): 2'-O-methyl modified RNA base

SEQ ID NO: 53 - DNA, 33 bp, Artificial Sequence; identical to SEQ ID NO: 51
  source: /note="Description of Artificial Sequence: Synthetic oligonucleotide"
  source: /note="Description of Combined DNA/RNA Molecule: Synthetic oligonucleotide"
  modified_base (24)..(33): 2'-O-methyl modified RNA base

SEQ ID NO: 54 - DNA, 33 bp, Artificial Sequence
  source: /note="Description of Artificial Sequence: Synthetic oligonucleotide"
  source: /note="Description of Combined DNA/RNA Molecule: Synthetic oligonucleotide"
  modified_base (25)..(33): 2'-O-methyl modified RNA base
tgactccatatggagtcacatggtucauucgug

SEQ ID NO: 55 - DNA, 33 bp, Artificial Sequence; identical to SEQ ID NO: 49
  source: /note="Description of Artificial Sequence: Synthetic oligonucleotide"
  source: /note="Description of Combined DNA/RNA Molecule: Synthetic oligonucleotide"
  modified_base (26)..(33): 2'-O-methyl modified RNA base

SEQ ID NO: 56 - DNA, 33 bp, Artificial Sequence; identical to SEQ ID NO: 49
  source: /note="Description of Artificial Sequence: Synthetic oligonucleotide"
  source: /note="Description of Combined DNA/RNA Molecule: Synthetic oligonucleotide"
  modified_base (27)..(33): 2'-O-methyl modified RNA base

SEQ ID NO: 57 - DNA, 33 bp, Artificial Sequence; identical to SEQ ID NO: 49
  source: /note="Description of Artificial Sequence: Synthetic oligonucleotide"
  source: /note="Description of Combined DNA/RNA Molecule: Synthetic oligonucleotide"
  modified_base (28)..(33): 2'-O-methyl modified RNA base

SEQ ID NO: 58 - DNA, 29 bp, Artificial Sequence
  source: /note="Description of Artificial Sequence: Synthetic primer"
  source: /note="Description of Combined DNA/RNA Molecule: Synthetic primer"
  modified_base (18)..(18): 2'-O-methyl modified RNA base
  modified_base (20)..(20): 2'-O-methyl modified RNA base
  modified_base (22)..(22): 2'-O-methyl modified RNA base
  modified_base (24)..(28): 2'-O-methyl modified RNA base
cgcggagtcctcgaactataagccacgca

SEQ ID NO: 59 - DNA, 32 bp, Artificial Sequence
  source: /note="Description of Artificial Sequence: Synthetic primer"
  source: /note="Description of Combined DNA/RNA Molecule: Synthetic primer"
  modified_base (19)..(19): 2'-O-methyl modified RNA base
  modified_base (21)..(21): 2'-O-methyl modified RNA base
  modified_base (23)..(23): 2'-O-methyl modified RNA base
  modified_base (25)..(25): 2'-O-methyl modified RNA base
  modified_base (27)..(31): 2'-O-methyl modified RNA base
cgcggagtccgcgtgtacagctccaccacaut

SEQ ID NO: 60 - DNA, 29 bp, Artificial Sequence
  source: /note="Description of Artificial Sequence: Synthetic primer"
  source: /note="Description of Combined DNA/RNA Molecule: Synthetic primer"
  modified_base (24)..(29): 2'-O-methyl modified RNA base
cgcggagtcctcgaactataagccacgca

SEQ ID NO: 61 - DNA, 32 bp, Artificial Sequence
  source: /note="Description of Artificial Sequence: Synthetic primer"
  source: /note="Description of Combined DNA/RNA Molecule: Synthetic primer"
  modified_base (27)..(32): 2'-O-methyl modified RNA base
cgcggagtccgcgtgtacagctccaccacauu